European Patent Application EP 4 296 286 A1, published December 27, 2023. Title: ANTI-GPRC5D×BCMA×CD3 TRISPECIFIC ANTIBODY AND USE THEREOF. Applicant: Innovent Biologics (Suzhou) Co., Ltd. The sequence listing filed with the application follows.

SEQUENCE LISTING (125 sequences)

SEQ ID NO: 1 - protein, 8 aa, artificial sequence
  synthetic
GFTFSSYG

SEQ ID NO: 2 - protein, 8 aa, artificial sequence
  synthetic
IWYDGSNK

SEQ ID NO: 3 - protein, 13 aa, artificial sequence
  synthetic
ARFTMFRGITLDY

SEQ ID NO: 4 - protein, 6 aa, artificial sequence
  synthetic
QRINSY

SEQ ID NO: 5 - protein, 3 aa, artificial sequence
  synthetic
ASS

SEQ ID NO: 6 - protein, 9 aa, artificial sequence
  synthetic
QQSYSTPLT

SEQ ID NO: 7 - protein, 9 aa, artificial sequence
  synthetic
GYSITSDYA

SEQ ID NO: 8 - protein, 7 aa, artificial sequence
  synthetic
IDYTGRT

SEQ ID NO: 9 - protein, 14 aa, artificial sequence
  synthetic
ARGNYGRYYYVMDY

SEQ ID NO: 10 - protein, 7 aa, artificial sequence
  synthetic
SQDIRNY

SEQ ID NO: 11 - protein, 3 aa, artificial sequence
  synthetic
YTS

SEQ ID NO: 12 - protein, 9 aa, artificial sequence
  synthetic
QQGNMLPWT

SEQ ID NO: 13 - protein, 10 aa, artificial sequence
  synthetic
GYTFIGYVMH

SEQ ID NO: 14 - protein, 17 aa, artificial sequence
  synthetic
YINPYNDVSQHQGKFKG

SEQ ID NO: 15 - protein, 11 aa, artificial sequence
  synthetic
EGRLGLRVLAY

SEQ ID NO: 16 - protein, 15 aa, artificial sequence
  synthetic
RASESVDSYGITFMN

SEQ ID NO: 17 - protein, 7 aa, artificial sequence
  synthetic
AASNQGS

SEQ ID NO: 18 - protein, 9 aa, artificial sequence
  synthetic
QQSKEVPWT

SEQ ID NO: 19 - protein, 10 aa, artificial sequence
  synthetic
GYTFTTYTMH

SEQ ID NO: 20 - protein, 17 aa, artificial sequence
  synthetic
FIIPSSGYTSYNQNFKD

SEQ ID NO: 21 - protein, 11 aa, artificial sequence
  synthetic
GQARAYYPLDY

SEQ ID NO: 22 - protein, 11 aa, artificial sequence
  synthetic
RASQSIGTTIH

SEQ ID NO: 23 - protein, 11 aa, artificial sequence
  synthetic
YASESISGIPS

SEQ ID NO: 24 - protein, 9 aa, artificial sequence
  synthetic
QQSYNWPRT

SEQ ID NO: 25 - protein, 120 aa, artificial sequence
  synthetic
QVQLVESGGGVVQPGRSLRLSCTASGFTFSSYGLHWVRQAPGKGLEWVAVIWYDGSNKYYIDSVKGRFIISRDNSKNTLYLQMNSLRAEDTAVYYCARFTMFRGITLDYWGQGTLVTVSS

SEQ ID NO: 26 - protein, 107 aa, artificial sequence
  synthetic
DIQMTQSPSSLSASVGDRVTITCRASQRINSYLNWYQQKPGKAPKLLIYAASSLQSGVPSRFSGSGSGTDFTLTISNLQPEDFATYYCQQSYSTPLTFGGGTKVEIK

SEQ ID NO: 27 - protein, 121 aa, artificial sequence
  synthetic
DVQLQESGPGLVKPSQSLSLTCTVTGYSITSDYAWNWIRQFPGNKLEWMVYIDYTGRTSYNPSLKSRISLTRDTSKNQFFLQFNSVTTEDTATYYCARGNYGRYYYVMDYWGQGTSVTVSS

SEQ ID NO: 28 - protein, 107 aa, artificial sequence
  synthetic
DIQMTQTTSSLSASLGDRVTISCRASQDIRNYLNWYQQRPDGTIKLLIYYTSRLHSGVPSRFSGSGSGTDYSLTISNLDQEDFATYFCQQGNMLPWTFGGGTSLEIK

SEQ ID NO: 29 - protein, 120 aa, artificial sequence
  synthetic
QVQLVQSGAEVKKPGASVKVSCKASGYTFIGYVMHWVRQAPGQGLEWMGYINPYNDVSQHQGKFKGRVTMTSDTSTSTVYMELSSLRSEDTAVYYCAREGRLGLRVLAYWGQGTLVTVSS

SEQ ID NO: 30 - protein, 111 aa, artificial sequence
  synthetic
DIVMTQSPDSLAVSLGERATINCRASESVDSYGITFMNWYQQKPGQPPKLLIYAASNQGSGVPDRFSGSGSGTDFTLTISSLQAEDVAVYYCQQSKEVPWTFGQGTKLEIK

SEQ ID NO: 31 - protein, 120 aa, artificial sequence
  synthetic
QVQLVQSGAEVKKPGSSVKVSCKASGYTFTTYTMHWVRQAPGQGLEWIGFIIPSSGYTSYNQNFKDKVTLTADKSTSTAYMELSSLRSEDTAVYFCTGGQARAYYPLDYWGQGTLVTVSS

SEQ ID NO: 32 - protein, 107 aa, artificial sequence
  synthetic
EIVMTQSPATLSVSPGERATLSCRASQSIGTTIHWYQQKPGQAPRLLIKYASESISGIPSRFSGSGSGTEFTLTISSLQSEDFAVYYCQQSYNWPRTFGGGTKVEIK

SEQ ID NO: 33 - protein, 10 aa, artificial sequence
  synthetic
GFTFGDYAIH

SEQ ID NO: 34 - protein, 17 aa, artificial sequence
  synthetic
GISWDSSSIAYADSVKG

SEQ ID NO: 35 - protein, 15 aa, artificial sequence
  synthetic
DSPVRDSFGSIAFDI

SEQ ID NO: 36 - protein, 11 aa, artificial sequence
  synthetic
RASQSVSSYLA

SEQ ID NO: 37 - protein, 7 aa, artificial sequence
  synthetic
DASKRAT

SEQ ID NO: 38 - protein, 9 aa, artificial sequence
  synthetic
QQASALPLT

SEQ ID NO: 39 - protein, 124 aa, artificial sequence
  synthetic
EVQLVESGGGLVQPGRSLRLSCAASGFTFGDYAIHWVRQAPGKGLEWVSGISWDSSSIAYADSVKGRFTISRDNAKNSLYLQMNSLRAEDTAVYYCAKDSPVRDSFGSIAFDIWGQGTMVTVSS

SEQ ID NO: 40 - protein, 107 aa, artificial sequence
  synthetic
EIVLTQSPATLSLSPGERATLSCRASQSVSSYLAWYQQKPGQAPRLLIYDASKRATGIPARFSGSGSGTDFTLTISSLEPEDFAVYYCQQASALPLTFGGGTKVEIK

SEQ ID NO: 41 - protein, 5 aa, artificial sequence
  synthetic
TYAMN

SEQ ID NO: 42 - protein, 19 aa, artificial sequence
  synthetic
RIRSKYNNYATYYADSVKD

SEQ ID NO: 43 - protein, 14 aa, artificial sequence
  synthetic
HGNFGQSYVSWFAY

SEQ ID NO: 44 - protein, 14 aa, artificial sequence
  synthetic
RSSTGAVTTSNYAN

SEQ ID NO: 45 - protein, 7 aa, artificial sequence
  synthetic
GTNKRAP

SEQ ID NO: 46 - protein, 9 aa, artificial sequence
  synthetic
ALWYSNLWV

SEQ ID NO: 47 - protein, 14 aa, artificial sequence
  synthetic
HYNFGQSYVSWFAY

SEQ ID NO: 48 - protein, 125 aa, artificial sequence
  synthetic
EVQLVESGGGLVQPGGSLKLSCAASGFTFNTYAMNWVRQASGKGLEWVGRIRSKYNNYATYYADSVKDRFTISRDDSKSTLYLQMNSLKTEDTAVYYCARHGNFGQSYVSWFAYWGQGTTVTVSS

SEQ ID NO: 49 - protein, 109 aa, artificial sequence
  synthetic
QAVVTQEPSLTVSPGGTVTLTCRSSTGAVTTSNYANWVQQKPGQAPRGLIGGTNKRAPGVPARFSGSLLGDKAALTLLGAQPEDEAEYYCALWYSNLWVFGQGTKLTVL

SEQ ID NO: 50 - protein, 125 aa, artificial sequence
  synthetic
EVQLVESGGGLVQPGGSLKLSCAASGFTFNTYAMNWVRQASGKGLEWVGRIRSKYNNYATYYADSVKDRFTISRDDSKSTLYLQMNSLKTEDTAVYYCARHYNFGQSYVSWFAYWGQGTTVTVSS

SEQ ID NO: 51 - protein, 20 aa, artificial sequence
  synthetic
GGGGSGGGGSGGGGSGGGGS

SEQ ID NO: 52 - protein, 10 aa, artificial sequence
  synthetic
GGGGSGGGGS

SEQ ID NO: 53 - protein, 15 aa, artificial sequence
  synthetic
GGGGSGGGGSGGGGS

SEQ ID NO: 54 - protein, 17 aa, artificial sequence
  synthetic
TSGGGGSGGGGSGGGGS

SEQ ID NO: 55 - protein, 247 aa, artificial sequence
  synthetic
DIQMTQSPSSLSASVGDRVTITCRASQRINSYLNWYQQKPGKAPKLLIYAASSLQSGVPSRFSGSGSGTDFTLTISNLQPEDFATYYCQQSYSTPLTFGCGTKVEIKGGGGSGGGGSGGGGSGGGGSQVQLVESGGGVVQPGRSLRLSCTASGFTFSSYGLHWVRQAPGKCLEWVAVIWYDGSNKYYIDSVKGRFIISRDNSKNTLYLQMNSLRAEDTAVYYCARFTMFRGITLDYWGQGTLVTVSS

SEQ ID NO: 56 - protein, 251 aa, artificial sequence
  synthetic
EIVLTQSPATLSLSPGERATLSCRASQSVSSYLAWYQQKPGQAPRLLIYDASKRATGIPARFSGSGSGTDFTLTISSLEPEDFAVYYCQQASALPLTFGCGTKVEIKGGGGSGGGGSGGGGSGGGGSEVQLVESGGGLVQPGRSLRLSCAASGFTFGDYAIHWVRQAPGKCLEWVSGISWDSSSIAYADSVKGRFTISRDNAKNSLYLQMNSLRAEDTAVYYCAKDSPVRDSFGSIAFDIWGQGTMVTVSS

SEQ ID NO: 57 - protein, 246 aa, artificial sequence
  synthetic
EIVLTQSPATLSLSPGERATLSCRASQSVSSYLAWYQQKPGQAPRLLIYDASKRATGIPARFSGSGSGTDFTLTISSLEPEDFAVYYCQQASALPLTFGCGTKVEIKGGGGSGGGGSGGGGSEVQLVESGGGLVQPGRSLRLSCAASGFTFGDYAIHWVRQAPGKCLEWVSGISWDSSSIAYADSVKGRFTISRDNAKNSLYLQMNSLRAEDTAVYYCAKDSPVRDSFGSIAFDIWGQGTMVTVSS

SEQ ID NO: 58 - protein, 254 aa, artificial sequence
  synthetic
QAVVTQEPSLTVSPGGTVTLTCRSSTGAVTTSNYANWVQQKPGQAPRGLIGGTNKRAPGVPARFSGSLLGDKAALTLLGAQPEDEAEYYCALWYSNLWVFGCGTKLTVLGGGGSGGGGSGGGGSGGGGSEVQLVESGGGLVQPGGSLKLSCAASGFTFNTYAMNWVRQASGKCLEWVGRIRSKYNNYATYYADSVKDRFTISRDDSKSTLYLQMNSLKTEDTAVYYCARHGNFGQSYVSWFAYWGQGTTVTVSS

SEQ ID NO: 59 - protein, 254 aa, artificial sequence
  synthetic
EVQLVESGGGLVQPGGSLKLSCAASGFTFNTYAMNWVRQASGKCLEWVGRIRSKYNNYATYYADSVKDRFTISRDDSKSTLYLQMNSLKTEDTAVYYCARHGNFGQSYVSWFAYWGQGTTVTVSSGGGGSGGGGSGGGGSGGGGSQAVVTQEPSLTVSPGGTVTLTCRSSTGAVTTSNYANWVQQKPGQAPRGLIGGTNKRAPGVPARFSGSLLGDKAALTLLGAQPEDEAEYYCALWYSNLWVFGCGTKLTVL

SEQ ID NO: 60 - protein, 248 aa, artificial sequence
  synthetic
DIQMTQTTSSLSASLGDRVTISCRASQDIRNYLNWYQQRPDGTIKLLIYYTSRLHSGVPSRFSGSGSGTDYSLTISNLDQEDFATYFCQQGNMLPWTFGCGTSLEIKGGGGSGGGGSGGGGSGGGGSDVQLQESGPGLVKPSQSLSLTCTVTGYSITSDYAWNWIRQFPGNCLEWMVYIDYTGRTSYNPSLKSRISLTRDTSKNQFFLQFNSVTTEDTATYYCARGNYGRYYYVMDYWGQGTSVTVSS

SEQ ID NO: 61 - protein, 479 aa, artificial sequence
  synthetic
DIQMTQSPSSLSASVGDRVTITCRASQRINSYLNWYQQKPGKAPKLLIYAASSLQSGVPSRFSGSGSGTDFTLTISNLQPEDFATYYCQQSYSTPLTFGCGTKVEIKGGGGSGGGGSGGGGSGGGGSQVQLVESGGGVVQPGRSLRLSCTASGFTFSSYGLHWVRQAPGKCLEWVAVIWYDGSNKYYIDSVKGRFIISRDNSKNTLYLQMNSLRAEDTAVYYCARFTMFRGITLDYWGQGTLVTVSSEPKSCDKTHTCPPCPAPEAAGGPSVFLFPPKPKDTLMISRTPEVTCVVVDVSHEDPEVKFNWYVDGVEVHNAKTKPREEQYNSTYRVVSVLTVLHQDWLNGKEYKCKVSNKALPAPIEKTISKAKGQPREPQVYTLPPSRDELTKNQVSLSCAVKGFYPSDIAVEWESNGQPENNYKTTPPVLDSDGSFFLVSKLTVDKSRWQQGNVFSCSVMHEALHNHYTQKSLSLSPGK

SEQ ID NO: 62 - protein, 747 aa, artificial sequence
  synthetic
QAVVTQEPSLTVSPGGTVTLTCRSSTGAVTTSNYANWVQQKPGQAPRGLIGGTNKRAPGVPARFSGSLLGDKAALTLLGAQPEDEAEYYCALWYSNLWVFGCGTKLTVLGGGGSGGGGSGGGGSGGGGSEVQLVESGGGLVQPGGSLKLSCAASGFTFNTYAMNWVRQASGKCLEWVGRIRSKYNNYATYYADSVKDRFTISRDDSKSTLYLQMNSLKTEDTAVYYCARHGNFGQSYVSWFAYWGQGTTVTVSSEPKSCDKTHTCPPCPAPEAAGGPSVFLFPPKPKDTLMISRTPEVTCVVVDVSHEDPEVKFNWYVDGVEVHNAKTKPREEQYNSTYRVVSVLTVLHQDWLNGKEYKCKVSNKALPAPIEKTISKAKGQPREPQVYTLPPSRDELTKNQVSLWCLVKGFYPSDIAVEWESNGQPENNYKTTPPVLDSDGSFFLYSKLTVDKSRWQQGNVFSCSVMHEALHNHYTQKSLSLSPGKGGGGSGGGGSEIVLTQSPATLSLSPGERATLSCRASQSVSSYLAWYQQKPGQAPRLLIYDASKRATGIPARFSGSGSGTDFTLTISSLEPEDFAVYYCQQASALPLTFGCGTKVEIKGGGGSGGGGSGGGGSGGGGSEVQLVESGGGLVQPGRSLRLSCAASGFTFGDYAIHWVRQAPGKCLEWVSGISWDSSSIAYADSVKGRFTISRDNAKNSLYLQMNSLRAEDTAVYYCAKDSPVRDSFGSIAFDIWGQGTMVTVSS

SEQ ID NO: 63 - protein, 483 aa, artificial sequence
  synthetic
EIVLTQSPATLSLSPGERATLSCRASQSVSSYLAWYQQKPGQAPRLLIYDASKRATGIPARFSGSGSGTDFTLTISSLEPEDFAVYYCQQASALPLTFGCGTKVEIKGGGGSGGGGSGGGGSGGGGSEVQLVESGGGLVQPGRSLRLSCAASGFTFGDYAIHWVRQAPGKCLEWVSGISWDSSSIAYADSVKGRFTISRDNAKNSLYLQMNSLRAEDTAVYYCAKDSPVRDSFGSIAFDIWGQGTMVTVSSEPKSCDKTHTCPPCPAPEAAGGPSVFLFPPKPKDTLMISRTPEVTCVVVDVSHEDPEVKFNWYVDGVEVHNAKTKPREEQYNSTYRVVSVLTVLHQDWLNGKEYKCKVSNKALPAPIEKTISKAKGQPREPQVYTLPPSRDELTKNQVSLSCAVKGFYPSDIAVEWESNGQPENNYKTTPPVLDSDGSFFLVSKLTVDKSRWQQGNVFSCSVMHEALHNHYTQKSLSLSPGK

SEQ ID NO: 64 - protein, 743 aa, artificial sequence
  synthetic
QAVVTQEPSLTVSPGGTVTLTCRSSTGAVTTSNYANWVQQKPGQAPRGLIGGTNKRAPGVPARFSGSLLGDKAALTLLGAQPEDEAEYYCALWYSNLWVFGCGTKLTVLGGGGSGGGGSGGGGSGGGGSEVQLVESGGGLVQPGGSLKLSCAASGFTFNTYAMNWVRQASGKCLEWVGRIRSKYNNYATYYADSVKDRFTISRDDSKSTLYLQMNSLKTEDTAVYYCARHGNFGQSYVSWFAYWGQGTTVTVSSEPKSCDKTHTCPPCPAPEAAGGPSVFLFPPKPKDTLMISRTPEVTCVVVDVSHEDPEVKFNWYVDGVEVHNAKTKPREEQYNSTYRVVSVLTVLHQDWLNGKEYKCKVSNKALPAPIEKTISKAKGQPREPQVYTLPPSRDELTKNQVSLWCLVKGFYPSDIAVEWESNGQPENNYKTTPPVLDSDGSFFLYSKLTVDKSRWQQGNVFSCSVMHEALHNHYTQKSLSLSPGKGGGGSGGGGSDIQMTQSPSSLSASVGDRVTITCRASQRINSYLNWYQQKPGKAPKLLIYAASSLQSGVPSRFSGSGSGTDFTLTISNLQPEDFATYYCQQSYSTPLTFGCGTKVEIKGGGGSGGGGSGGGGSGGGGSQVQLVESGGGVVQPGRSLRLSCTASGFTFSSYGLHWVRQAPGKCLEWVAVIWYDGSNKYYIDSVKGRFIISRDNSKNTLYLQMNSLRAEDTAVYYCARFTMFRGITLDYWGQGTLVTVSS

SEQ ID NO: 65 - protein, 450 aa, artificial sequence
  synthetic
QVQLVESGGGVVQPGRSLRLSCTASGFTFSSYGLHWVRQAPGKGLEWVAVIWYDGSNKYYIDSVKGRFIISRDNSKNTLYLQMNSLRAEDTAVYYCARFTMFRGITLDYWGQGTLVTVSSASTKGPSVFPLAPSSKSTSGGTAALGCLVKDYFPEPVTVSWNSGALTSGVHTFPAVLQSSGLYSLSSVVTVPSSSLGTQTYICNVNHKPSNTKVDKKVEPKSCDKTHTCPPCPAPEAAGGPSVFLFPPKPKDTLMISRTPEVTCVVVDVSHEDPEVKFNWYVDGVEVHNAKTKPREEQYNSTYRVVSVLTVLHQDWLNGKEYKCKVSNKALPAPIEKTISKAKGQPREPQVYTLPPSRDELTKNQVSLSCAVKGFYPSDIAVEWESNGQPENNYKTTPPVLDSDGSFFLVSKLTVDKSRWQQGNVFSCSVMHEALHNHYTQKSLSLSPGK

SEQ ID NO: 66 - protein, 214 aa, artificial sequence
  synthetic
DIQMTQSPSSLSASVGDRVTITCRASQRINSYLNWYQQKPGKAPKLLIYAASSLQSGVPSRFSGSGSGTDFTLTISNLQPEDFATYYCQQSYSTPLTFGGGTKVEIKRTVAAPSVFIFPPSDEQLKSGTASVVCLLNNFYPREAKVQWKVDNALQSGNSQESVTEQDSKDSTYSLSSTLTLSKADYEKHKVYACEVTHQGLSSPVTKSFNRGEC

SEQ ID NO: 67 - protein, 716 aa, artificial sequence
  synthetic
EVQLVESGGGLVQPGGSLKLSCAASGFTFNTYAMNWVRQASGKGLEWVGRIRSKYNNYATYYADSVKDRFTISRDDSKSTLYLQMNSLKTEDTAVYYCARHGNFGQSYVSWFAYWGQGTTVTVSSASTKGPSVFPLAPSSKSTSGGTAALGCLVKDYFPEPVTVSWNSGALTSGVHTFPAVLQSSGLYSLSSVVTVPSSSLGTQTYICNVNHKPSNTKVDKKVEPKSCDKTHTCPPCPAPEAAGGPSVFLFPPKPKDTLMISRTPEVTCVVVDVSHEDPEVKFNWYVDGVEVHNAKTKPREEQYNSTYRVVSVLTVLHQDWLNGKEYKCKVSNKALPAPIEKTISKAKGQPREPQVYTLPPSRDELTKNQVSLWCLVKGFYPSDIAVEWESNGQPENNYKTTPPVLDSDGSFFLYSKLTVDKSRWQQGNVFSCSVMHEALHNHYTQKSLSLSPGKGGGGSGGGGSEIVLTQSPATLSLSPGERATLSCRASQSVSSYLAWYQQKPGQAPRLLIYDASKRATGIPARFSGSGSGTDFTLTISSLEPEDFAVYYCQQASALPLTFGCGTKVEIKGGGGSGGGGSGGGGSGGGGSEVQLVESGGGLVQPGRSLRLSCAASGFTFGDYAIHWVRQAPGKCLEWVSGISWDSSSIAYADSVKGRFTISRDNAKNSLYLQMNSLRAEDTAVYYCAKDSPVRDSFGSIAFDIWGQGTMVTVSS

SEQ ID NO: 68 - protein, 215 aa, artificial sequence
  synthetic
QAVVTQEPSLTVSPGGTVTLTCRSSTGAVTTSNYANWVQQKPGQAPRGLIGGTNKRAPGVPARFSGSLLGDKAALTLLGAQPEDEAEYYCALWYSNLWVFGQGTKLTVLGQPKAAPSVTLFPPSSEELQANKATLVCLISDFYPGAVTVAWKADSSPVKAGVETTTPSKQSNNKYAASSYLSLTPEQWKSHRSYSCQVTHEGSTVEKTVAPTECS

SEQ ID NO: 69 - protein, 454 aa, artificial sequence
  synthetic
EVQLVESGGGLVQPGRSLRLSCAASGFTFGDYAIHWVRQAPGKGLEWVSGISWDSSSIAYADSVKGRFTISRDNAKNSLYLQMNSLRAEDTAVYYCAKDSPVRDSFGSIAFDIWGQGTMVTVSSASTKGPSVFPLAPSSKSTSGGTAALGCLVKDYFPEPVTVSWNSGALTSGVHTFPAVLQSSGLYSLSSVVTVPSSSLGTQTYICNVNHKPSNTKVDKKVEPKSCDKTHTCPPCPAPEAAGGPSVFLFPPKPKDTLMISRTPEVTCVVVDVSHEDPEVKFNWYVDGVEVHNAKTKPREEQYNSTYRVVSVLTVLHQDWLNGKEYKCKVSNKALPAPIEKTISKAKGQPREPQVYTLPPSRDELTKNQVSLSCAVKGFYPSDIAVEWESNGQPENNYKTTPPVLDSDGSFFLVSKLTVDKSRWQQGNVFSCSVMHEALHNHYTQKSLSLSPGK

SEQ ID NO: 70 - protein, 214 aa, artificial sequence
  synthetic
EIVLTQSPATLSLSPGERATLSCRASQSVSSYLAWYQQKPGQAPRLLIYDASKRATGIPARFSGSGSGTDFTLTISSLEPEDFAVYYCQQASALPLTFGGGTKVEIKRTVAAPSVFIFPPSDEQLKSGTASVVCLLNNFYPREAKVQWKVDNALQSGNSQESVTEQDSKDSTYSLSSTLTLSKADYEKHKVYACEVTHQGLSSPVTKSFNRGEC

SEQ ID NO: 71 - protein, 712 aa, artificial sequence
  synthetic
EVQLVESGGGLVQPGGSLKLSCAASGFTFNTYAMNWVRQASGKGLEWVGRIRSKYNNYATYYADSVKDRFTISRDDSKSTLYLQMNSLKTEDTAVYYCARHGNFGQSYVSWFAYWGQGTTVTVSSASTKGPSVFPLAPSSKSTSGGTAALGCLVKDYFPEPVTVSWNSGALTSGVHTFPAVLQSSGLYSLSSVVTVPSSSLGTQTYICNVNHKPSNTKVDKKVEPKSCDKTHTCPPCPAPEAAGGPSVFLFPPKPKDTLMISRTPEVTCVVVDVSHEDPEVKFNWYVDGVEVHNAKTKPREEQYNSTYRVVSVLTVLHQDWLNGKEYKCKVSNKALPAPIEKTISKAKGQPREPQVYTLPPSRDELTKNQVSLWCLVKGFYPSDIAVEWESNGQPENNYKTTPPVLDSDGSFFLYSKLTVDKSRWQQGNVFSCSVMHEALHNHYTQKSLSLSPGKGGGGSGGGGSDIQMTQSPSSLSASVGDRVTITCRASQRINSYLNWYQQKPGKAPKLLIYAASSLQSGVPSRFSGSGSGTDFTLTISNLQPEDFATYYCQQSYSTPLTFGCGTKVEIKGGGGSGGGGSGGGGSGGGGSQVQLVESGGGVVQPGRSLRLSCTASGFTFSSYGLHWVRQAPGKCLEWVAVIWYDGSNKYYIDSVKGRFIISRDNSKNTLYLQMNSLRAEDTAVYYCARFTMFRGITLDYWGQGTLVTVSS

SEQ ID NO: 72 - protein, 451 aa, artificial sequence
  synthetic
DVQLQESGPGLVKPSQSLSLTCTVTGYSITSDYAWNWIRQFPGNKLEWMVYIDYTGRTSYNPSLKSRISLTRDTSKNQFFLQFNSVTTEDTATYYCARGNYGRYYYVMDYWGQGTSVTVSSASTKGPSVFPLAPSSKSTSGGTAALGCLVKDYFPEPVTVSWNSGALTSGVHTFPAVLQSSGLYSLSSVVTVPSSSLGTQTYICNVNHKPSNTKVDKKVEPKSCDKTHTCPPCPAPEAAGGPSVFLFPPKPKDTLMISRTPEVTCVVVDVSHEDPEVKFNWYVDGVEVHNAKTKPREEQYNSTYRVVSVLTVLHQDWLNGKEYKCKVSNKALPAPIEKTISKAKGQPREPQVYTLPPSRDELTKNQVSLSCAVKGFYPSDIAVEWESNGQPENNYKTTPPVLDSDGSFFLVSKLTVDKSRWQQGNVFSCSVMHEALHNHYTQKSLSLSPGK

SEQ ID NO: 73 - protein, 214 aa, artificial sequence
  synthetic
DIQMTQTTSSLSASLGDRVTISCRASQDIRNYLNWYQQRPDGTIKLLIYYTSRLHSGVPSRFSGSGSGTDYSLTISNLDQEDFATYFCQQGNMLPWTFGGGTSLEIKRTVAAPSVFIFPPSDEQLKSGTASVVCLLNNFYPREAKVQWKVDNALQSGNSQESVTEQDSKDSTYSLSSTLTLSKADYEKHKVYACEVTHQGLSSPVTKSFNRGEC

SEQ ID NO: 74 - protein, 711 aa, artificial sequence
  synthetic
EVQLVESGGGLVQPGGSLKLSCAASGFTFNTYAMNWVRQASGKGLEWVGRIRSKYNNYATYYADSVKDRFTISRDDSKSTLYLQMNSLKTEDTAVYYCARHGNFGQSYVSWFAYWGQGTTVTVSSASTKGPSVFPLAPSSKSTSGGTAALGCLVKDYFPEPVTVSWNSGALTSGVHTFPAVLQSSGLYSLSSVVTVPSSSLGTQTYICNVNHKPSNTKVDKKVEPKSCDKTHTCPPCPAPEAAGGPSVFLFPPKPKDTLMISRTPEVTCVVVDVSHEDPEVKFNWYVDGVEVHNAKTKPREEQYNSTYRVVSVLTVLHQDWLNGKEYKCKVSNKALPAPIEKTISKAKGQPREPQVYTLPPSRDELTKNQVSLWCLVKGFYPSDIAVEWESNGQPENNYKTTPPVLDSDGSFFLYSKLTVDKSRWQQGNVFSCSVMHEALHNHYTQKSLSLSPGKGGGGSGGGGSEIVLTQSPATLSLSPGERATLSCRASQSVSSYLAWYQQKPGQAPRLLIYDASKRATGIPARFSGSGSGTDFTLTISSLEPEDFAVYYCQQASALPLTFGCGTKVEIKGGGGSGGGGSGGGGSEVQLVESGGGLVQPGRSLRLSCAASGFTFGDYAIHWVRQAPGKCLEWVSGISWDSSSIAYADSVKGRFTISRDNAKNSLYLQMNSLRAEDTAVYYCAKDSPVRDSFGSIAFDIWGQGTMVTVSS

SEQ ID NO: 75 - protein, 450 aa, artificial sequence
  synthetic
QVQLVQSGAEVKKPGASVKVSCKASGYTFIGYVMHWVRQAPGQGLEWMGYINPYNDVSQHQGKFKGRVTMTSDTSTSTVYMELSSLRSEDTAVYYCAREGRLGLRVLAYWGQGTLVTVSSASTKGPSVFPLAPSSKSTSGGTAALGCLVKDYFPEPVTVSWNSGALTSGVHTFPAVLQSSGLYSLSSVVTVPSSSLGTQTYICNVNHKPSNTKVDKKVEPKSCDKTHTCPPCPAPEAAGGPSVFLFPPKPKDTLMISRTPEVTCVVVDVSHEDPEVKFNWYVDGVEVHNAKTKPREEQYNSTYRVVSVLTVLHQDWLNGKEYKCKVSNKALPAPIEKTISKAKGQPREPQVYTLPPSRDELTKNQVSLWCLVKGFYPSDIAVEWESNGQPENNYKTTPPVLDSDGSFFLYSKLTVDKSRWQQGNVFSCSVMHEALHNHYTQKSLSLSPGK

SEQ ID NO: 76 - protein, 218 aa, artificial sequence
  synthetic
DIVMTQSPDSLAVSLGERATINCRASESVDSYGITFMNWYQQKPGQPPKLLIYAASNQGSGVPDRFSGSGSGTDFTLTISSLQAEDVAVYYCQQSKEVPWTFGQGTKLEIKRTVAAPSVFIFPPSDEQLKSGTASVVCLLNNFYPREAKVQWKVDNALQSGNSQESVTEQDSKDSTYSLSSTLTLSKADYEKHKVYACEVTHQGLSSPVTKSFNRGEC

SEQ ID NO: 77 - protein, 711 aa, artificial sequence
  synthetic
EVQLVESGGGLVQPGGSLKLSCAASGFTFNTYAMNWVRQASGKGLEWVGRIRSKYNNYATYYADSVKDRFTISRDDSKSTLYLQMNSLKTEDTAVYYCARHGNFGQSYVSWFAYWGQGTTVTVSSASTKGPSVFPLAPSSKSTSGGTAALGCLVKDYFPEPVTVSWNSGALTSGVHTFPAVLQSSGLYSLSSVVTVPSSSLGTQTYICNVNHKPSNTKVDKKVEPKSSDKTHTCPPCPAPEAAGGPSVFLFPPKPKDTLMISRTPEVTCVVVDVSHEDPEVKFNWYVDGVEVHNAKTKPREEQYNSTYRVVSVLTVLHQDWLNGKEYKCKVSNKALPAPIEKTISKAKGQPREPQVYTLPPSRDELTKNQVSLSCAVKGFYPSDIAVEWESNGQPENNYKTTPPVLDSDGSFFLVSKLTVDKSRWQQGNVFSCSVMHEALHNHYTQKSLSLSPGKGGGGSGGGGSEIVLTQSPATLSLSPGERATLSCRASQSVSSYLAWYQQKPGQAPRLLIYDASKRATGIPARFSGSGSGTDFTLTISSLEPEDFAVYYCQQASALPLTFGCGTKVEIKGGGGSGGGGSGGGGSEVQLVESGGGLVQPGRSLRLSCAASGFTFGDYAIHWVRQAPGKCLEWVSGISWDSSSIAYADSVKGRFTISRDNAKNSLYLQMNSLRAEDTAVYYCAKDSPVRDSFGSIAFDIWGQGTMVTVSS

SEQ ID NO: 78 - protein, 711 aa, artificial sequence
  synthetic
EVQLVESGGGLVQPGGSLKLSCAASGFTFNTYAMNWVRQASGKGLEWVGRIRSKYNNYATYYADSVKDRFTISRDDSKSTLYLQMNSLKTEDTAVYYCARHYNFGQSYVSWFAYWGQGTTVTVSSASTKGPSVFPLAPSSKSTSGGTAALGCLVKDYFPEPVTVSWNSGALTSGVHTFPAVLQSSGLYSLSSVVTVPSSSLGTQTYICNVNHKPSNTKVDKKVEPKSSDKTHTCPPCPAPEAAGGPSVFLFPPKPKDTLMISRTPEVTCVVVDVSHEDPEVKFNWYVDGVEVHNAKTKPREEQYNSTYRVVSVLTVLHQDWLNGKEYKCKVSNKALPAPIEKTISKAKGQPREPQVYTLPPSRDELTKNQVSLSCAVKGFYPSDIAVEWESNGQPENNYKTTPPVLDSDGSFFLVSKLTVDKSRWQQGNVFSCSVMHEALHNHYTQKSLSLSPGKGGGGSGGGGSEIVLTQSPATLSLSPGERATLSCRASQSVSSYLAWYQQKPGQAPRLLIYDASKRATGIPARFSGSGSGTDFTLTISSLEPEDFAVYYCQQASALPLTFGCGTKVEIKGGGGSGGGGSGGGGSEVQLVESGGGLVQPGRSLRLSCAASGFTFGDYAIHWVRQAPGKCLEWVSGISWDSSSIAYADSVKGRFTISRDNAKNSLYLQMNSLRAEDTAVYYCAKDSPVRDSFGSIAFDIWGQGTMVTVSS

SEQ ID NO: 79 - protein, 450 aa, artificial sequence
  synthetic
QVQLVQSGAEVKKPGSSVKVSCKASGYTFTTYTMHWVRQAPGQGLEWIGFIIPSSGYTSYNQNFKDKVTLTADKSTSTAYMELSSLRSEDTAVYFCTGGQARAYYPLDYWGQGTLVTVSSASTKGPSVFPLAPSSKSTSGGTAALGCLVKDYFPEPVTVSWNSGALTSGVHTFPAVLQSSGLYSLSSVVTVPSSSLGTQTYICNVNHKPSNTKVDKKVEPKSCDKTHTCPPCPAPEAAGGPSVFLFPPKPKDTLMISRTPEVTCVVVDVSHEDPEVKFNWYVDGVEVHNAKTKPREEQYNSTYRVVSVLTVLHQDWLNGKEYKCKVSNKALPAPIEKTISKAKGQPREPQVYTLPPSRDELTKNQVSLWCLVKGFYPSDIAVEWESNGQPENNYKTTPPVLDSDGSFFLYSKLTVDKSRWQQGNVFSCSVMHEALHNHYTQKSLSLSPGK

SEQ ID NO: 80 - protein, 214 aa, artificial sequence
  synthetic
EIVMTQSPATLSVSPGERATLSCRASQSIGTTIHWYQQKPGQAPRLLIKYASESISGIPSRFSGSGSGTEFTLTISSLQSEDFAVYYCQQSYNWPRTFGGGTKVEIKRTVAAPSVFIFPPSDEQLKSGTASVVCLLNNFYPREAKVQWKVDNALQSGNSQESVTEQDSKDSTYSLSSTLTLSKADYEKHKVYACEVTHQGLSSPVTKSFNRGEC

SEQ ID NO: 81 - protein, 712 aa, artificial sequence
  synthetic
DVQLQESGPGLVKPSQSLSLTCTVTGYSITSDYAWNWIRQFPGNKLEWMVYIDYTGRTSYNPSLKSRISLTRDTSKNQFFLQFNSVTTEDTATYYCARGNYGRYYYVMDYWGQGTSVTVSSASTKGPSVFPLAPSSKSTSGGTAALGCLVKDYFPEPVTVSWNSGALTSGVHTFPAVLQSSGLYSLSSVVTVPSSSLGTQTYICNVNHKPSNTKVDKKVEPKSCDKTHTCPPCPAPEAAGGPSVFLFPPKPKDTLMISRTPEVTCVVVDVSHEDPEVKFNWYVDGVEVHNAKTKPREEQYNSTYRVVSVLTVLHQDWLNGKEYKCKVSNKALPAPIEKTISKAKGQPREPQVYTLPPSRDELTKNQVSLTCLVKGFYPSDIAVEWESNGQPENNYKTTPPVLDSDGSFFLYSKLTVDKSRWQQGNVFSCSVMHEALHNHYTQKSLSLSPGKGGGGSGGGGSEIVLTQSPATLSLSPGERATLSCRASQSVSSYLAWYQQKPGQAPRLLIYDASKRATGIPARFSGSGSGTDFTLTISSLEPEDFAVYYCQQASALPLTFGCGTKVEIKGGGGSGGGGSGGGGSGGGGSEVQLVESGGGLVQPGRSLRLSCAASGFTFGDYAIHWVRQAPGKCLEWVSGISWDSSSIAYADSVKGRFTISRDNAKNSLYLQMNSLRAEDTAVYYCAKDSPVRDSFGSIAFDIWGQGTMVTVSS

SEQ ID NO: 82 - protein, 478 aa, artificial sequence
  synthetic
DIQMTQTTSSLSASLGDRVTISCRASQDIRNYLNWYQQRPDGTIKLLIYYTSRLHSGVPSRFSGSGSGTDYSLTISNLDQEDFATYFCQQGNMLPWTFGGGTSLEIKRTVAAPSVFIFPPSDEQLKSGTASVVCLLNNFYPREAKVQWKVDNALQSGNSQESVTEQDSKDSTYSLSSTLTLSKADYEKHKVYACEVTHQGLSSPVTKSFNRGECGGGGSGGGGSQAVVTQEPSLTVSPGGTVTLTCRSSTGAVTTSNYANWVQQKPGQAPRGLIGGTNKRAPGVPARFSGSLLGDKAALTLLGAQPEDEAEYYCALWYSNLWVFGCGTKLTVLGGGGSGGGGSGGGGSGGGGSEVQLVESGGGLVQPGGSLKLSCAASGFTFNTYAMNWVRQASGKCLEWVGRIRSKYNNYATYYADSVKDRFTISRDDSKSTLYLQMNSLKTEDTAVYYCARHGNFGQSYVSWFAYWGQGTTVTVSS

SEQ ID NO: 83 - protein, 478 aa, artificial sequence
  synthetic
DIQMTQTTSSLSASLGDRVTISCRASQDIRNYLNWYQQRPDGTIKLLIYYTSRLHSGVPSRFSGSGSGTDYSLTISNLDQEDFATYFCQQGNMLPWTFGGGTSLEIKRTVAAPSVFIFPPSDEQLKSGTASVVCLLNNFYPREAKVQWKVDNALQSGNSQESVTEQDSKDSTYSLSSTLTLSKADYEKHKVYACEVTHQGLSSPVTKSFNRGECGGGGSGGGGSEVQLVESGGGLVQPGGSLKLSCAASGFTFNTYAMNWVRQASGKCLEWVGRIRSKYNNYATYYADSVKDRFTISRDDSKSTLYLQMNSLKTEDTAVYYCARHGNFGQSYVSWFAYWGQGTTVTVSSGGGGSGGGGSGGGGSGGGGSQAVVTQEPSLTVSPGGTVTLTCRSSTGAVTTSNYANWVQQKPGQAPRGLIGGTNKRAPGVPARFSGSLLGDKAALTLLGAQPEDEAEYYCALWYSNLWVFGCGTKLTVL

SEQ ID NO: 84 - protein, 712 aa, artificial sequence
  synthetic
EVQLVESGGGLVQPGRSLRLSCAASGFTFGDYAIHWVRQAPGKGLEWVSGISWDSSSIAYADSVKGRFTISRDNAKNSLYLQMNSLRAEDTAVYYCAKDSPVRDSFGSIAFDIWGQGTMVTVSSASTKGPSVFPLAPSSKSTSGGTAALGCLVKDYFPEPVTVSWNSGALTSGVHTFPAVLQSSGLYSLSSVVTVPSSSLGTQTYICNVNHKPSNTKVDKKVEPKSSDKTHTCPPCPAPELLGGPSVFLFPPKPKDTLMISRTPEVTCVVVDVSHEDPEVKFNWYVDGVEVHNAKTKPREEQYNSTYRVVSVLTVLHQDWLNGKEYKCKVSNKALPAPIEKTISKAKGQPREPQVYTLPPSRDELTKNQVSLTCLVKGFYPSDIAVEWESNGQPENNYKTTPPVLDSDGSFFLYSKLTVDKSRWQQGNVFSCSVMHEALHNHYTQKSLSLSPGKGGGGSGGGGSDIQMTQTTSSLSASLGDRVTISCRASQDIRNYLNWYQQRPDGTIKLLIYYTSRLHSGVPSRFSGSGSGTDYSLTISNLDQEDFATYFCQQGNMLPWTFGCGTSLEIKGGGGSGGGGSGGGGSGGGGSDVQLQESGPGLVKPSQSLSLTCTVTGYSITSDYAWNWIRQFPGNCLEWMVYIDYTGRTSYNPSLKSRISLTRDTSKNQFFLQFNSVTTEDTATYYCARGNYGRYYYVMDYWGQGTSVTVSS

SEQ ID NO: 85 - protein, 478 aa, artificial sequence
  synthetic
EIVLTQSPATLSLSPGERATLSCRASQSVSSYLAWYQQKPGQAPRLLIYDASKRATGIPARFSGSGSGTDFTLTISSLEPEDFAVYYCQQASALPLTFGGGTKVEIKRTVAAPSVFIFPPSDEQLKSGTASVVCLLNNFYPREAKVQWKVDNALQSGNSQESVTEQDSKDSTYSLSSTLTLSKADYEKHKVYACEVTHQGLSSPVTKSFNRGECGGGGSGGGGSQAVVTQEPSLTVSPGGTVTLTCRSSTGAVTTSNYANWVQQKPGQAPRGLIGGTNKRAPGVPARFSGSLLGDKAALTLLGAQPEDEAEYYCALWYSNLWVFGCGTKLTVLGGGGSGGGGSGGGGSGGGGSEVQLVESGGGLVQPGGSLKLSCAASGFTFNTYAMNWVRQASGKCLEWVGRIRSKYNNYATYYADSVKDRFTISRDDSKSTLYLQMNSLKTEDTAVYYCARHGNFGQSYVSWFAYWGQGTTVTVSS

SEQ ID NO: 86 - protein, 478 aa, artificial sequence
  synthetic
EIVLTQSPATLSLSPGERATLSCRASQSVSSYLAWYQQKPGQAPRLLIYDASKRATGIPARFSGSGSGTDFTLTISSLEPEDFAVYYCQQASALPLTFGGGTKVEIKRTVAAPSVFIFPPSDEQLKSGTASVVCLLNNFYPREAKVQWKVDNALQSGNSQESVTEQDSKDSTYSLSSTLTLSKADYEKHKVYACEVTHQGLSSPVTKSFNRGECGGGGSGGGGSEVQLVESGGGLVQPGGSLKLSCAASGFTFNTYAMNWVRQASGKCLEWVGRIRSKYNNYATYYADSVKDRFTISRDDSKSTLYLQMNSLKTEDTAVYYCARHGNFGQSYVSWFAYWGQGTTVTVSSGGGGSGGGGSGGGGSGGGGSQAVVTQEPSLTVSPGGTVTLTCRSSTGAVTTSNYANWVQQKPGQAPRGLIGGTNKRAPGVPARFSGSLLGDKAALTLLGAQPEDEAEYYCALWYSNLWVFGCGTKLTVL

SEQ ID NO: 87 - protein, 450 aa, artificial sequence; identical to SEQ ID NO: 75
  synthetic

SEQ ID NO: 88 - protein, 481 aa, artificial sequence
  synthetic
DIVMTQSPDSLAVSLGERATINCRASESVDSYGITFMNWYQQKPGQPPKLLIYAASNQGSGVPDRFSGSGSGTDFTLTISSLQAEDVAVYYCQQSKEVPWTFGQGTKLEIKRTVAAPSVFIFPPSDEQLKSGTASVVCLLNNFYPREAKVQWKVDNALQSGNSQESVTEQDSKDSTYSLSSTLTLSKADYEKHKVYACEVTHQGLSSPVTKSFNRGECTSGGGGSGGGGSGGGGSEIVLTQSPATLSLSPGERATLSCRASQSVSSYLAWYQQKPGQAPRLLIYDASKRATGIPARFSGSGSGTDFTLTISSLEPEDFAVYYCQQASALPLTFGCGTKVEIKGGGGSGGGGSGGGGSEVQLVESGGGLVQPGRSLRLSCAASGFTFGDYAIHWVRQAPGKCLEWVSGISWDSSSIAYADSVKGRFTISRDNAKNSLYLQMNSLRAEDTAVYYCAKDSPVRDSFGSIAFDIWGQGTMVTVSS

SEQ ID NO: 89 - protein, 478 aa, artificial sequence
  synthetic
QAVVTQEPSLTVSPGGTVTLTCRSSTGAVTTSNYANWVQQKPGQAPRGLIGGTNKRAPGVPARFSGSLLGDKAALTLLGAQPEDEAEYYCALWYSNLWVFGQGTKLTVLGQPKAAPSVTLFPPSSEELQANKATLVCLISDFYPGAVTVAWKADSSPVKAGVETTTPSKQSNNKYAASSYLSLTPEQWKSHRSYSCQVTHEGSTVEKTVAPTECSTSGGGGSGGGGSGGGGSEIVLTQSPATLSLSPGERATLSCRASQSVSSYLAWYQQKPGQAPRLLIYDASKRATGIPARFSGSGSGTDFTLTISSLEPEDFAVYYCQQASALPLTFGCGTKVEIKGGGGSGGGGSGGGGSEVQLVESGGGLVQPGRSLRLSCAASGFTFGDYAIHWVRQAPGKCLEWVSGISWDSSSIAYADSVKGRFTISRDNAKNSLYLQMNSLRAEDTAVYYCAKDSPVRDSFGSIAFDIWGQGTMVTVSS

SEQ ID NO: 90 - protein, 450 aa, artificial sequence; identical to SEQ ID NO: 79
  synthetic

SEQ ID NO: 91 - protein, 477 aa, artificial sequence
  synthetic
EIVMTQSPATLSVSPGERATLSCRASQSIGTTIHWYQQKPGQAPRLLIKYASESISGIPSRFSGSGSGTEFTLTISSLQSEDFAVYYCQQSYNWPRTFGGGTKVEIKRTVAAPSVFIFPPSDEQLKSGTASVVCLLNNFYPREAKVQWKVDNALQSGNSQESVTEQDSKDSTYSLSSTLTLSKADYEKHKVYACEVTHQGLSSPVTKSFNRGECTSGGGGSGGGGSGGGGSEIVLTQSPATLSLSPGERATLSCRASQSVSSYLAWYQQKPGQAPRLLIYDASKRATGIPARFSGSGSGTDFTLTISSLEPEDFAVYYCQQASALPLTFGCGTKVEIKGGGGSGGGGSGGGGSEVQLVESGGGLVQPGRSLRLSCAASGFTFGDYAIHWVRQAPGKCLEWVSGISWDSSSIAYADSVKGRFTISRDNAKNSLYLQMNSLRAEDTAVYYCAKDSPVRDSFGSIAFDIWGQGTMVTVSS

SEQ ID NO: 92 - protein, 451 aa, artificial sequence
  synthetic
DVQLQESGPGLVKPSQSLSLTCTVTGYSITSDYAWNWIRQFPGNKLEWMVYIDYTGRTSYNPSLKSRISLTRDTSKNQFFLQFNSVTTEDTATYYCARGNYGRYYYVMDYWGQGTSVTVSSASTKGPSVFPLAPSSKSTSGGTAALGCLVKDYFPEPVTVSWNSGALTSGVHTFPAVLQSSGLYSLSSVVTVPSSSLGTQTYICNVNHKPSNTKVDKKVEPKSCDKTHTCPPCPAPEAAGGPSVFLFPPKPKDTLMISRTPEVTCVVVDVSHEDPEVKFNWYVDGVEVHNAKTKPREEQYNSTYRVVSVLTVLHQDWLNGKEYKCKVSNKALPAPIEKTISKAKGQPREPQVYTLPPSRDELTKNQVSLWCLVKGFYPSDIAVEWESNGQPENNYKTTPPVLDSDGSFFLYSKLTVDKSRWQQGNVFSCSVMHEALHNHYTQKSLSLSPGK

SEQ ID NO: 93 - protein, 478 aa, artificial sequence; identical to SEQ ID NO: 82
  synthetic

SEQ ID NO: 94 - protein, 454 aa, artificial sequence; identical to SEQ ID NO: 69
  synthetic

SEQ ID NO: 95 - protein, 478 aa, artificial sequence; identical to SEQ ID NO: 85
  synthetic

SEQ ID NO: 96 - protein, 478 aa, artificial sequence; identical to SEQ ID NO: 83
  synthetic

SEQ ID NO: 97 - protein, 478 aa, artificial sequence; identical to SEQ ID NO: 86
  synthetic

SEQ ID NO: 98 - protein, 120 aa, artificial sequence
  synthetic
EVQLQQSGPELVKPGASVKMSCKASGYTFIGYVMHWVKRKPGQGLEWIGYINPYNDVSQHNGKFKGKATLTSDKSSSTAYMELSSLTSEDSAVYYCAREGRLGLRVLAYWGQGTLVTVSA

SEQ ID NO: 99 - protein, 111 aa, artificial sequence
  synthetic
DIVLTQSPASLAVSLGQRATISCRASESVDSYGITFMNWFQQKPGQPPKLLIYAASNQGSGVPARFSGSGSGTDFSLNIHPMEEDDTAMYFCQQSKEVPWTFGGGTKLEIK

SEQ ID NO: 100 - protein, 120 aa, artificial sequence
  synthetic
EVQLQQSVAELARPGASVKMSCKASGYTFTTYTMHWVKQRPGQGLEWIGFIIPSSGYTSYNQNFKDKVTLTADKSSSTAYMQLSSLTSEDSAVYFCTGGQARAYYPLDYWGQGTSVTVSS

SEQ ID NO: 101 - protein, 107 aa, artificial sequence
  synthetic
DIVMTQSPAILSVSPGERVSFSCRASQSIGTTIHWYQQRSNGSPRLLIKYASESISGIPSRFSGSGSGTYFTLSINSVESEDIADYFCQQSYNWPRTFGGGTKLEIK

SEQ ID NO: 102 - protein, 232 aa, artificial sequence
  synthetic
EPKSCDKTHTCPPCPAPEAAGGPSVFLFPPKPKDTLMISRTPEVTCVVVDVSHEDPEVKFNWYVDGVEVHNAKTKPREEQYNSTYRVVSVLTVLHQDWLNGKEYKCKVSNKALPAPIEKTISKAKGQPREPQVYTLPPSRDELTKNQVSLSCAVKGFYPSDIAVEWESNGQPENNYKTTPPVLDSDGSFFLVSKLTVDKSRWQQGNVFSCSVMHEALHNHYTQKSLSLSPGK

SEQ ID NO: 103 - protein, 232 aa, artificial sequence
  synthetic
EPKSCDKTHTCPPCPAPEAAGGPSVFLFPPKPKDTLMISRTPEVTCVVVDVSHEDPEVKFNWYVDGVEVHNAKTKPREEQYNSTYRVVSVLTVLHQDWLNGKEYKCKVSNKALPAPIEKTISKAKGQPREPQVYTLPPSRDELTKNQVSLWCLVKGFYPSDIAVEWESNGQPENNYKTTPPVLDSDGSFFLYSKLTVDKSRWQQGNVFSCSVMHEALHNHYTQKSLSLSPGK

SEQ ID NO: 104 - protein, 98 aa, artificial sequence
  synthetic
ASTKGPSVFPLAPSSKSTSGGTAALGCLVKDYFPEPVTVSWNSGALTSGVHTFPAVLQSSGLYSLSSVVTVPSSSLGTQTYICNVNHKPSNTKVDKKV

SEQ ID NO: 105 - protein, 107 aa, artificial sequence [sequence omitted]

SEQ ID NO: 106 - protein, 106 aa, artificial sequence
  synthetic
GQPKAAPSVTLFPPSSEELQANKATLVCLISDFYPGAVTVAWKADSSPVKAGVETTTPSKQSNNKYAASSYLSLTPEQWKSHRSYSCQVTHEGSTVEKTVAPTECS

SEQ ID NO: 107 - protein, 232 aa, artificial sequence
  synthetic
EPKSSDKTHTCPPCPAPEAAGGPSVFLFPPKPKDTLMISRTPEVTCVVVDVSHEDPEVKFNWYVDGVEVHNAKTKPREEQYNSTYRVVSVLTVLHQDWLNGKEYKCKVSNKALPAPIEKTISKAKGQPREPQVYTLPPSRDELTKNQVSLSCAVKGFYPSDIAVEWESNGQPENNYKTTPPVLDSDGSFFLVSKLTVDKSRWQQGNVFSCSVMHEALHNHYTQKSLSLSPGK

SEQ ID NO: 108 - protein, 232 aa, artificial sequence
  synthetic
EPKSCDKTHTCPPCPAPEAAGGPSVFLFPPKPKDTLMISRTPEVTCVVVDVSHEDPEVKFNWYVDGVEVHNAKTKPREEQYNSTYRVVSVLTVLHQDWLNGKEYKCKVSNKALPAPIEKTISKAKGQPREPQVYTLPPSRDELTKNQVSLTCLVKGFYPSDIAVEWESNGQPENNYKTTPPVLDSDGSFFLYSKLTVDKSRWQQGNVFSCSVMHEALHNHYTQKSLSLSPGK

SEQ ID NO: 109 - protein, 232 aa, artificial sequence
  synthetic
EPKSSDKTHTCPPCPAPELLGGPSVFLFPPKPKDTLMISRTPEVTCVVVDVSHEDPEVKFNWYVDGVEVHNAKTKPREEQYNSTYRVVSVLTVLHQDWLNGKEYKCKVSNKALPAPIEKTISKAKGQPREPQVYTLPPSRDELTKNQVSLTCLVKGFYPSDIAVEWESNGQPENNYKTTPPVLDSDGSFFLYSKLTVDKSRWQQGNVFSCSVMHEALHNHYTQKSLSLSPGK

SEQ ID NO: 110 - protein, 17 aa, artificial sequence
  synthetic
YINPYNDVSQHNGKFKG

SEQ ID NO: 111 - protein, 454 aa, artificial sequence
  synthetic
EVQLVESGGGLVQPGRSLRLSCAASGFTFGDYAIHWVRQAPGKGLEWVSGISWDSSSIAYADSVKGRFTISRDNAKNSLYLQMNSLRAEDTAVYYCAKDSPVRDSFGSIAFDIWGQGTMVTVSSASTKGPSVFPLAPSSKSTSGGTAALGCLVKDYFPEPVTVSWNSGALTSGVHTFPAVLQSSGLYSLSSVVTVPSSSLGTQTYICNVNHKPSNTKVDKKVEPKSCDKTHTCPPCPAPEAAGGPSVFLFPPKPKDTLMISRTPEVTCVVVDVSHEDPEVKFNWYVDGVEVHNAKTKPREEQYNSTYRVVSVLTVLHQDWLNGKEYKCKVSNKALPAPIEKTISKAKGQPREPQVYTLPPCRDELTKNQVSLWCLVKGFYPSDIAVEWESNGQPENNYKTTPPVLDSDGSFFLYSKLTVDKSRWQQGNVFSCSVMHEALHNHYTQKSLSLSPGK

SEQ ID NO: 112 - protein, 214 aa, artificial sequence; identical to SEQ ID NO: 70
  synthetic

SEQ ID NO: 113 - protein, 485 aa, artificial sequence
  synthetic
DIVMTQSPDSLAVSLGERATINCKSSQSLLNARTGKNYLAWYQQKPGQPPKLLIYWASTRESGVPDRFSGSGSGTDFTLTISSLQAEDVAVYYCKQSYSRRTFGCGTKVEIKGGGGSGGGGSGGGGSGGGGSQVQLVQSGAEVKKPGASVKVSCKASGFNIKDYYMHWVRQAPGQCLEWMGWIDLENANTVYNAKFQGRVTITRDTSASTAYMELSSLRSEDTAVYYCARDAYGRYFYDVWGQGTLVTVSSGSEPKSSDKTHTCPPCPAPEAAGGPSVFLFPPKPKDTLMISRTPEVTCVVVDVSHEDPEVKFNWYVDGVEVHNAKTKPREEQYNSTYRVVSVLTVLHQDWLNGKEYKCKVSNKALPAPIEKTISKAKGQPREPQVCTLPPSRDELTKNQVSLSCAVKGFYPSDIAVEWESNGQPENNYKTTPPVLDSDGSFFLVSKLTVDKSRWQQGNVFSCSVMHEALHNHYTQKSLSLSPGK

SEQ ID NO: 114 - protein, 15 aa, artificial
  synthetic
EPKSCDKTHTCPPCP

SEQ ID NO: 115 - protein, 15 aa, artificial
  synthetic
EPKSSDKTHTCPPCP

SEQ ID NO: 116 - protein, 3 aa, artificial
  sythetic
GGG

SEQ ID NO: 117 - protein, 5 aa, artificial
  synthetic
DGGGS

SEQ ID NO: 118 - protein, 5 aa, artificial
  synthetic
TGEKP

SEQ ID NO: 119 - protein, 4 aa, artificial
  synthetic
GGRR

SEQ ID NO: 120 - protein, 14 aa, artificial
  synthetic
EGKSSGSGSESKVD

SEQ ID NO: 121 - protein, 18 aa, artificial
  synthetic
KESGSVSSEQLAQFRSLD

SEQ ID NO: 122 - protein, 8 aa, artificial
  synthetic
GGRRGGGS

SEQ ID NO: 123 - protein, 9 aa, artificial
  synthetic
LRQRDGERP

SEQ ID NO: 124 - protein, 12 aa, artificial
  synthetic
LRQKDGGGSERP

SEQ ID NO: 125 - protein, 18 aa, artificial
  synthetic
GSTSGSGKPGSGEGSTKG